European Patent Application EP 4 782 534 A1, published July 29, 2026. Title: 一种修饰细胞的方法及其应用. Applicant: 北京领新博瑞生物科技有限公司. Application WO. The sequence listing filed with the application follows.

SEQUENCE LISTING (13 sequences)

SEQ ID NO: 1 - protein, 7 aa, synthetic construct
  REGION 1..7: note = CD20 antibody HCDR1
GYTFTSY

SEQ ID NO: 2 - protein, 5 aa, synthetic construct
  REGION 1..5: note = CD20 antibody HCDR2
PGNGD

SEQ ID NO: 3 - protein, 12 aa, synthetic construct
  REGION 1..12: note = CD20 antibody HCDR3
STYYGGDWYFNV

SEQ ID NO: 4 - protein, 121 aa, synthetic construct
  REGION 1..121: note = CD20 antibody VH
QVQLQQPGAELVKPGASVKMSCKASGYTFTSYNMHWVKQTPGRGLEWIGAIYPGNGDTSYNQKFKGKATLTADKSSSTAYMQLSSLTSEDSAVYYCARSTYYGGDWYFNVWGAGTTVTVSS

SEQ ID NO: 5 - protein, 10 aa, synthetic construct
  REGION 1..10: note = CD20 antibody LCDR1
RASSSVSYIH

SEQ ID NO: 6 - protein, 7 aa, synthetic construct
  REGION 1..7: note = CD20 antibody LCDR2
ATSNLAS

SEQ ID NO: 7 - protein, 9 aa, synthetic construct
  REGION 1..9: note = CD20 antibody LCDR3
QQWTSNPPT

SEQ ID NO: 8 - protein, 108 aa, synthetic construct
  REGION 1..108: note = CD20 antibody VL
QIVLSQSPAILSASPGEKVTMTCRASSSVSYIHWFQQKPGSSPKPWIYATSNLASGVPVRFSGSGSGTSYSLTISRVEAEDAATYYCQQWTSNPPTFGGGTKLEIKRT

SEQ ID NO: 9 - protein, 7 aa, synthetic construct
  REGION 1..7: note = Claudin 18.2 antibody HCDR1
VDISSDV

SEQ ID NO: 10 - protein, 8 aa, synthetic construct
  REGION 1..8: note = Claudin 18.2 antibody HCDR2
LTRGGSIN

SEQ ID NO: 11 - protein, 14 aa, synthetic construct
  REGION 1..14: note = Claudin 18.2 antibody HCDR3
NAEIYTGTFYPRSY

SEQ ID NO: 12 - protein, 120 aa, synthetic construct
  REGION 1..120: note = Claudin 18.2 nanobody VH
QLQLVESGGGLVQPGGSLRLSCAASGVDISSDVMAWYRQAPGKQREFVSGLTRGGSINYADSVKGRFTISRDFAKNTVDLQMNSIKPEDTAVYYCNAEIYTGTFYPRSYWGQGTQVTVSS

SEQ ID NO: 13 - protein, 352 aa, synthetic construct
  REGION 1..352: note = Claudin 18.2 nanobody VHH-Fc
QLQLVESGGGLVQPGGSLRLSCAASGVDISSDVMAWYRQAPGKQREFVSGLTRGGSINYADSVKGRFTISRDFAKNTVDLQMNSIKPEDTAVYYCNAEIYTGTFYPRSYWGQGTQVTVSSEPKSADKTHTCPPCPAPELLGGPSVFLFPPKPKDTLMISRTPEVTCVVVDVSHEDPEVKFNWYVDGVEVHNAKTKPREEQYNSTYRVVSVLTVLHQDWLNGKEYKCKVSNKALPAPIEKTISKAKGQPREPQVYTLPPSREEMTKNQVSLTCLVKGFYPSDIAVEWESNGQPENNYKTTPPVLDSDGSFFLYSKLTVDKSRWQQGNVFSCSVMHEALHNHYTQKSLSLSPGK